European Patent Specification EP 4 330 424 B1, published March 12, 2025. Title: AMPLIFICATION OF SINGLE STRANDED DNA. Applicant: • THE UNIVERSITY COURT OF THE UNIVERSITY OF EDINBURGH. The sequence listing filed with the application follows.

SEQUENCE LISTING (8 sequences)

SEQ ID NO: 1 - DNA, 21 bp, Artificial Sequence
  primer
ggcaatgaagtcgcagggttg

SEQ ID NO: 2 - DNA, 22 bp, Artificial Sequence
  primer
aagcagtggtatcaacgcagag

SEQ ID NO: 3 - DNA, 40 bp, Artificial Sequence
  oligonucleotide
atagcgttgataccactgcttctcacgacagactcgctaa

SEQ ID NO: 4 - DNA, 25 bp, Artificial Sequence
  oligonucleotide
tggactgatgcgagtctgtcgtgag

SEQ ID NO: 5 - DNA, 38 bp, Artificial Sequence
  oligonucleotide
aatgacgctggacgaacacggcaatgaagtcgcagaca

SEQ ID NO: 6 - DNA, 27 bp, Artificial Sequence
  oligonucleotide
gtgttcgtccagcgtccaggtgagtgg

SEQ ID NO: 7 - DNA, 27 bp, Artificial Sequence
  primer
ccactcacctggacgctggacgaacac

SEQ ID NO: 8 - DNA, 59 bp, Artificial Sequence
  template
  misc_structure 23: /note="Single stranded cDNA template: i.e. 5’-3’ – sequence of 5’ pre-attached adapter, sequence of cDNA represented by N and sequence of 3’ pre-attached adapter"
aagcagtggtatcaacgcagagnnnnnnnnnnnnnnnncaaccctgcgacttcattgcc